European Patent Application EP 4 506 356 A1, published February 12, 2025. Title: METHANOL-INDUCIBLE PROMOTER AND USE THEREOF IN PREPARATION OF L-ALANYL-L-GLUTAMINE. Applicant: WUHAN GRAND HOYO CO., LTD. The sequence listing filed with the application follows.

SEQUENCE LISTING (25 sequences)

SEQ ID NO: 1 - DNA, 1099 bp, Artificial Sequence
  Promoter sequence of gene PpRNA_RS07685
aatgatatttgagggtgttagttacttcgtctccagagtagcttatagggagaaaaaccgagacaacgatggaactcccatgtagattccaccgccccaattactgttttgggcaatcctgttgataagacgcattctagagttgtttcatgaaagggttacgggtgttgattggtttgagatatgccagaggacagatcaatctgtggtttgctaaactggaagtctggtaaggactctagcaagtccgttactcaaaaagtcataccaagtaagattacgtaacacctgggcatgactttctaagttagcaagtcaccaagagggtcctatttaacgtttggcggtatctgaaacacaagacttgcctatcccatagtacatcatattacctgtcaagctatgctaccccacagaaataccccaaaagttgaagtgaaaaaatgaaaattactggtaacttcaccccataacaaacttaataatttctgtagccaatgaaagtaaaccccattcaatgttccgagatttagtatacttgcccctataagaaacgaaggatttcagcttccttaccccatgaacagaaatcttccatttaccccccactggagagatccgcccaaacgaacagataatagaaaaaagaaattcggacaaatagaacactttctcagccaattaaagtcattccatgcactccctttagctgccgttccatccctttgttgagcaacaccatcgttagccagtacgaaagaggaaacttaaccgataccttggagaaatctaaggcgcgaatgagtttagcctagatatccttagtgaagggttgttccgatacttctccacattcagtcatagatgggcagctttgttatcatgaagagacggaaacgggcattaagggttaaccgccaaattatataaagacaacatgtccccagtttaaagtttttctttcctattcttgtatcctgagtgaccgttgtgtttaatataacaagttcgttttaacttaagaccaaaaccagttacaacaaattataacccctctaaacactaaagttcactcttatcaaactatcaaacatcaaaa

SEQ ID NO: 2 - DNA, 397 bp, Artificial Sequence
  Promoter sequence of gene PpRNA_RS11281
gatgagtatcaaaggggatttggttatgcgatgcaacgagagattgtttatcccagatgctgatgtaaaaaccttaaccagcgtgacagtagaaataagacacgttaaaattacccgcgcttccctaacaattggctctgcctttcggcaagtttctaactgccctcccctctcacatgcaccacgaacttaccgttcgctcctagcagaaccaccccaaagtttaatcaggaccgcattttagcctattgctgtagaaccccacaacataacctggtccagagccagccctttatatatggtaaatcccgtttgaacttcgaagtggaatcggaatttttacatcaaagaaactgatactgaaacttttggcttcgacttggactttctcttaatc

SEQ ID NO: 3 - DNA, 458 bp, Artificial Sequence
  Promoter sequence of gene PpRNA_RS05760
gtctttgtaaatagttatagttcagaaactggaattgagctcaaaaaactggaatcgagcggatatttgaagattgatgccttactcatgaattgattgataagagctccgtgattcactctgtcaatgattacccctctcctacccgatttgggactttttcttcagtcttggggactttttttcatatgacttgaccttgctttcccaatagggaaggactcacccatggatgattaagtttggattactcgtttaggaaatagtagccatgaatcaatttgaatcataccatcatgaaatagggttaggctgtaaatgcctcaaaaatggctcttgaggctggatttttgggtattggaatgttggtagcaattggtataaaaggccatttgtatttcacttttttgtccttcatactttactcttctcaactttggaaacttcaataaatcatc

SEQ ID NO: 4 - DNA, 1529 bp, Artificial Sequence
  Promoter sequence of gene PpRNA_RS04123
gaattctttttttcagaccatatgaccggtccatcttctacggggggattatctatgctttgacctctatcttgattcttttatgattcaaatcacttttacgttatttattacttactggttatttacttagcgccttttctgaaaaacatttactaaaaatcatacatcggcactctcaaacacgacagattgtgatcaagaagcagagacaatcaccactaaggttgcacatttgagccagtaggctcctaatagaggttcgatacttattttgataatacgacatattgtcttacctctgaatgtgtcaatactctctcgttcttcgtctcgtcagctaaaaatataacacttcgagtaagatacgcccaattgaaggctacgagataccagactatcactagtagaactttgacatctgctaaagcagatcaaatatccatttatccagaatcaattaccttcctttagcttgtcgaaggcatgaaaaagctacatgaaaatccccatccttgaagttttgtcagcttaaaggactccatttcctaaaatttcaagcagtcctctcaactaaatttttttccattcctctgcacccagccctcttcatcaaccgtccagccttctcaaaagtccaatgtaagtagcctgcaaattcaggttacaacccctcaattttccatccaagggcgatccttacaaagttaatatcgaacagcagagactaagcgagtcatcatcaccacccaacgatggtgaaaaactttaagcatagattgatggagggtgtatggcacttggcggctgcattagagtttgaaactatggggtaatacatcacatccggaactgatccgactccgagatcatatgcaaagcacgtgatgtaccccgtaaactgctcggattatcgttgcaattcatcgtcttaaacagtacaagaaactttattcatgggtcattggactctgatgaggggcacatttccccaatgattttttgggaaagaaagccgtaagaggacagttaagcgaaagagacaagacaacgaacagcaaaagtgacagctgtcagctacctagtggacagttgggagtttccaattggttggttttgaatttttacccatgttgagttgtccttgcttctccttgcaaacaatgcaagttgataagacatcaccttccaagataggctatttttgtcgcataaatttttgtctcggagtgaaaaccccttttatgtgaacagattacagaagcgtcctacccttcaccggttgagatggggagaaaattaagcgatgaggagacgattattggtataaaagaagcaaccaaaatcccttattgtccttttctgatcagcatcaaagaatattgtcttaaaacgggcttttaactacattgttcttacacattgcaaacctcttccttctatttcggatcaactgtattgactacattgatcttttttaacgaagtttacgacttactaaatccccacaaacaaatcaactgagaaaa

SEQ ID NO: 5 - DNA, 366 bp, Artificial Sequence
  Promoter sequence of gene PpRNA_RS00891
gaattagtgagataacagagttgggtaactagagagaataatagacgtatgcatgattactacacaacggatgtcgcactctttccttagttaaaactatcatccaatcacaagatgcgggctggaaagacttgctcccgaaggataatcttctgcttctatctcccttcctcatatggtttcgcagggctcatgccccttcttccttcgaactgcccgatgaggaagtccttagcctatcaaagaattcgggaccatcatcgatttttagagccttacctgatcgcaatcaggatttcactactcatataaatacatcgctcaaagctccaactttgcttgttcatacaattcttgatattcaca

SEQ ID NO: 6 - DNA, 480 bp, Artificial Sequence
  Promoter sequence of gene PpRNA_RS02207
ttctggagtgtcaaaacagtagtgataaaaggctatgaaggaggttgtctaggggctcgtggaggaaagtgattcaaacagacctgccaaaaagagaaaaaagagggaatccctgttctttccaatggaaatgacgtaactttgacttgaaaaataccccaaccagaagggttcaaactcaacaaggattgcgtaattcctacaagtagcttagagctgggggagagacaactgaaggcagcttaacgataactcggggggattggtgcacgactcgaaaggaggtttcttagtcttgtaacctcttttttccagaggctattcaagattcataggcgatatcgatgtggagaagggtgaacaatataaaaggctggagagatgtcaatgaagcggctggatagatttcaaattttctagatttcagagtaatcgcacaaaacgaaggaatcacaccaagacaaaaaaaaaaattctaag

SEQ ID NO: 7 - DNA, 26 bp, Artificial Sequence
  PpRNA_RS07685Fp primer sequence
aatgatatttgagggtgttagttact

SEQ ID NO: 8 - DNA, 31 bp, Artificial Sequence
  PpRNA_RS07685Rp primer sequence
ttttgatgtttgatagtttgataagagtgaa

SEQ ID NO: 9 - DNA, 25 bp, Artificial Sequence
  PpRNA_RS11281Fp primer sequence
gatgagtatcaaaggggatttggtt

SEQ ID NO: 10 - DNA, 25 bp, Artificial Sequence
  PpRNA_RS11281Rp primer sequence
gattaagagaaagtccaagtcgaag

SEQ ID NO: 11 - DNA, 32 bp, Artificial Sequence
  PpRNA_RS05760Fp primer sequence
gtctttgtaaatagttatagttcagaaactgg

SEQ ID NO: 12 - DNA, 30 bp, Artificial Sequence
  PpRNA_RS05760Rp primer sequence
gatgatttattgaagtttccaaagttgaga

SEQ ID NO: 13 - DNA, 28 bp, Artificial Sequence
  PpRNA_RS04123Fp primer sequence
gaattctttttttcagaccatatgaccg

SEQ ID NO: 14 - DNA, 25 bp, Artificial Sequence
  PpRNA_RS04123Rp primer sequence
ttttctcagttgatttgtttgtggg

SEQ ID NO: 15 - DNA, 27 bp, Artificial Sequence
  PpRNA_RS00891Fp primer sequence
gaattagtgagataacagagttgggta

SEQ ID NO: 16 - DNA, 31 bp, Artificial Sequence
  PpRNA_RS00891Rp primer sequence
tgtgaatatcaagaattgtatgaacaagcaa

SEQ ID NO: 17 - DNA, 26 bp, Artificial Sequence
  PpRNA_RS02207Fp primer sequence
ttctggagtgtcaaaacagtagtgat

SEQ ID NO: 18 - DNA, 29 bp, Artificial Sequence
  PpRNA_RS02207Rp primer sequence
cttagaatttttttttttgtcttggtggg

SEQ ID NO: 19 - DNA, 31 bp, Artificial Sequence
  SAETFp primer sequence
ccggaattcatgactcgaagaggtggttccg

SEQ ID NO: 20 - DNA, 36 bp, Artificial Sequence
  SAETRP primer sequence
aaatatgcggccgcaggctgaatcacaggaaggtca

SEQ ID NO: 21 - DNA, 25 bp, Artificial Sequence
  gapRT-Fp primer sequence
ggtattaacggtttcggacgtattg

SEQ ID NO: 22 - DNA, 25 bp, Artificial Sequence
  gapRT-Rp primer sequence
gatgttgacagggtctctctcttgg

SEQ ID NO: 23 - DNA, 23 bp, Artificial Sequence
  SAetRT-Fp primer sequence
ggtatccatgctgcctggtttac

SEQ ID NO: 24 - DNA, 23 bp, Artificial Sequence
  SAetRT-Rp
gcgatctgatggacgtcgtagtt

SEQ ID NO: 25 - DNA, 1860 bp, Artificial Sequence
  AET nucleotide sequence
atgaaaaatacaatttcgtgcctaactttagcgcttttaagcgcaagccagttacatgctcaaacagctgccgactcggcttatgttagagatcattatgaaaagaccgaagtagcaattcccatgcgagatgggaaaaaattatttactgcgatctacagtccaaaagacaaatccaagaaatatccagttttgctcaatagaacgccctacacggtttctccttatgggcagaacgaatacaaaaaaagtttgggaaactttccccaaatgatgcgtgaaggctatattttcgtttaccaggatgtccgtggcaagtggatgagcgaaggtgattttgaagatatacgtccgaccacgtacagcaaagataaaaaagcaatcgatgaaagtacggatacctatgatgcgcttgaatggttacagaaaaatctcaaaaactataatggcaaagccgggctctatgggatttcctatccaggcttctattctaccgtcggattggtcaaaacacacccgagcttgaaggcagtctccccacaggctcccgtaacagactggtatatcggcgacgacttccaccataatggcgtattgtttcttcaggatgcatttacattcatgtcaacctttggtgtccctcgtccaaaacccattacaccggatcaatttaagggcaaaattcagatcaaagaagccgataaatataacttttttgcagaagcaggaacagcgcgggaactcaaagaaaaatactttggtgactccgtacaattttggaatgacctgtttaagcatcccgactatgatgatttttggaaatcgcgtgtgatcaccaattctttacaggaggtaaaaccagctgtgatggtggttggtggtttctttgacgcggaagatgcttatggaacatttaagacctaccaatcgattgaggataaaagcaaaaaaaacaactcgattttagtcgcgggaccttggtatcatggcggctgggttcgtgcagaaggaaactatttaggtgatatccaatttgagaaaaaaaccagtattacttatcaggaacaatttgaacaaccgtttttcaaatattacctaaaagatgaaggaaacttcgccccttccgaagccaacatttttgtttcaggcagcaacgaatggaaacatttcgaacaatggccaccaaaaaatgtagagacaaaaaaactatacttccaacctcaggggaaacttggatttgacaaagttcaacgtacagattcctgggatgaatatgtaacagacccgaataaacctgttccgcatcaaggtgggttaattcaaaaccgaacacgggagtatatggtagatgatcaacgtttcgcggctagtcgccctgatgtcatggtttatcaaacggaaccgttgacggaggacctgacgatagtaggcccaatcaaaaactttctcaaagtttcttcaacaggaacagacgcggactatgttgtcaaactgattgacgtttatccgaatgatgcagcaagttatcaaggaaaaacaatggctggatatcaaatgatggtacgtggtgagatcatggcggggaaataccgaaatggtttcgataaagcgcaggccttgactccaggtatggtcgaaaaggtgaattttgaaatgccagacgttgcgcataccttcaaaaaaggacatcgcattatggttcaggtacaaaactcatggtttccgctggcagaacgaaatccacaggtgtttttagcaccttatacagctaccaaagctgatttccgcaaagctacccaacgtatttttcacgatgtgaacaatgccacatacatcgaattttctgtcctcaaagattag